European Patent Application EP 4 643 876 A1, published November 5, 2025. Title: PHARMACEUTICAL PREPARATION COMPRISING ANTI-TIGIT ANTIBODY. Applicant: Shanghai Henlius Biotech, Inc. Application CN. The sequence listing filed with the application follows.

SEQUENCE LISTING (2 sequences)

SEQ ID NO: 1 - protein, 125 aa, synthetic construct
  source 1..125: note = VHH
QVQLVESGGGVVQPGRSLRLSCAASGGSFSSYPMGWFRQAPGKERESVAAISSDLRFTYYADSVKGRFTISRDNSKNTLYLQMNSLRAEDTAVYYCAARTSGVGYYSRAQWYDYWGQGTLVTVSS

SEQ ID NO: 2 - protein, 357 aa, synthetic construct
  source 1..357: note = heavy chain
QVQLVESGGGVVQPGRSLRLSCAASGGSFSSYPMGWFRQAPGKERESVAAISSDLRFTYYADSVKGRFTISRDNSKNTLYLQMNSLRAEDTAVYYCAARTSGVGYYSRAQWYDYWGQGTLVTVSSEPKSCDKTHTCPPCPAPELLGGPSVFLFPPKPKDTLMISRTPEVTCVVVDVSHEDPEVKFNWYVDGVEVHNAKTKPREEQYNSTYRVVSVLTVLHQDWLNGKEYKCKVSNKALPAPIEKTISKAKGQPREPQVYTLPPSREEMTKNQVSLTCLVKGFYPSDIAVEWESNGQPENNYKTTPPVLDSDGSFFLYSKLTVDKSRWQQGNVFSCSVMHEALHNHYTQKSLSLSPGK